European Patent Specification EP 3 679 131 B1, published September 4, 2024. Title: Leistungsverbesserte Proteasevarianten II. Applicant: Henkel AG & Co. KGaA. The sequence listing filed with the application follows.

SEQUENCE LISTING (24 sequences)

SEQ ID NO: 1 - protein, 275 aa, Bacillus pumilus
AQTVPYGIPQIKAPAVHAQGYKGANVKVAVLDTGIHAAHPDLNVAGGASFVPSEPNATQDFQSHGTHVAGTIAALDNTIGVLGVAPSASLYAVKVLDRNGDGQYSWIISGIEWAVANNMDVINMSLGGPNGSTALKNAVDTANNRGVVVVAAAGNSGSTGSTSTVGYPAKYDSTIAVANVNSSNVRNSSSSAGPELDVSAPGTSILSTVPSSGYTSYTGTSMASPHVAGAAALILSKNPNLSNSQVRQRLENTATPLGNSFYYGKGLINAQAASN

SEQ ID NO: 2 - protein, 275 aa, Artificial Sequence
  Ausgangsmutante 2
AQTVPYGITQIKAPAVHAQGYKGANVKVAVLDTGIHAAHPDLNVAGGASFVPSEPNATQDFQSHGTHVAGTIAALDNTIGVLGVAPSASLYAVKVLDRNGDGQYSWIISGIEWAVANNMDVINMSLGGPNGSRALKNAVDTANNRGVVVVAAAGNSGSTGSTSTVGYPAKYDSTIAVANVNSSNVRNSSSSAGPELDVSAPGTSILSTVPSSGYTCYTGTSMAAPHVAGAAALILSKNPNLSNSQVRQRLENTATPLGNSFYYGKGLINAEAASN

SEQ ID NO: 3 - protein, 275 aa, Artificial Sequence
  Mutationsvariante 1
AQTVPYGITQIKAPAVHAQGYKGANVKVAVLDTGIHAAHPDLNVAGGASFVPSEPNATQDFQSHGTHVAGTIAALDNTIGVLGVAPSASLYAVKVLDRNGDGQYSWIISGIEWAVANNMDVINMSLGGPDSSYALKNAVDTANNRGVVVVAAAGNSGSTGSTSTVGYPAKYDSTIAVANVNSSNVRNSSSSAGPELDVSAPGTSILSTVPSSGYTCYTGTSMAAPHVAGAAALILSKNPNLSNSQVRQRLENTATPLGNSFYYGKGLINAEAASN

SEQ ID NO: 4 - protein, 275 aa, Artificial Sequence
  Mutationsvariante 2
AQTVPYGITQIKAPAVHAQGYKGANVKVAVLDTGIHAAHPDLNVAGGASFVPSEPNATQDFQSHGTHVAGTIAALDNTIGVLGVAPSASLYAVKVLDRNGDGQYSWIISGIEWAVANNMDVINMSLGGPSSSYALKNAVDTANLRGVVVVAAAGNSGSTGSTSTVGYPAKYDSTIAVANVNSSNVRNSSSSAGPELDVSAPGTSILSTVPSSGYTCYTGTSMAAPHVAGAAALILSKNPNLSNSQVRQRLENTATPLGNSFYYGKGLINAEAASN

SEQ ID NO: 5 - protein, 275 aa, Artificial Sequence
  Mutationsvariante 3
AQTVPYGITQIKAPAVHAQGYKGANVKVAVLDTGIHAAHPDLNVAGGASFVPSEPNATQDFQSHGTHVAGTIAALDNTIGVLGVAPSASLYAVKVLDRNGDGQYSWIISGIEWAVANNMDVINMSLGGPDNSKALKNAVDTANKRGVVVVAAAGNSGSTGSTSTVGYPAKYDSTIAVANVNSSNVRNSSSSAGPELDVSAPGTSILSTVPSSGYTCYTGTSMASPHVAGAAALILSKNPNLSNSQVRQRLENTATPLGNSFYYGKGLINAEAASN

SEQ ID NO: 6 - protein, 275 aa, Artificial Sequence
  Mutationsvariante 4
AQTVPYGITQIKAPAVHAQGYKGANVKVAVLDTGIHAAHPDLNVAGGASFVPSEPNATQDFQSHGTHVAGTIAALDNTIGVLGVAPSASLYAVKVLDRNGDGQYSWIISGIEWAVANNMDVINMSLGGPHNSTALKNAVDTANKRGVVVVAAAGNSGSTGSTSTVGYPAKYDSTIAVANVNSSNVRNSSSSAGPELDVSAPGTSILSTVPSSGYTCYTGTSMAAPHVAGAAALILSKNPNLSNSQVRQRLENTATPLGNSFYYGKGLINAEAASN

SEQ ID NO: 7 - protein, 275 aa, Artificial Sequence
  Mutationsvariante 5
AQTVPYGITQIKAPAVHAQGYKGANVKVGVLDTGIHAAHPDLNVAGGASFVPSEPNATQDFQSHGTHVAGTIAALDNTIGVLGVAPSASLYAVKVLDRNGDGQYSWIISGIEWAVANNMDVINMSLGGPDNSRALKNAVDTANNRGVVVVAAAGNSGSTGSTSTVGYPAKYDSTIAVANVNSSNVRNSSSSAGPELDVSAPGTSILSTVPSSGYTCYTGTSMASPHVAGAAALILSKNPNLSNSQVRQRLENTATPLGNSFYYGKGLINAEAASN

SEQ ID NO: 8 - protein, 275 aa, Artificial Sequence
  Mutationsvariante 6
AQTVPYGITQIKAPAVHAQGYKGANVKVGVLDTGIHAAHPDLNVAGGASFVPSEPNATQDFQSHGTHVAGTIAALDNTIGVLGVAPSASLYAVKVLDRNGEGQYSWIISGIEWAVANNMDVINMSLGGPSSSTALKNAVDTANNRGVVVVAAAGNSGSTGSTSTVGYPAKYDSTIAVANVNSSNVRNSSSSAGPELDVSAPGTSILSTVPSSGYTCYTGTSMATPHVAGAAALILSKNPNLSNSQVRQRLESTATPLGNSFYYGKGLINAEAASN

SEQ ID NO: 9 - protein, 275 aa, Artificial Sequence
  Mutationsvariante 7
AQTVPYGITQIKAPAVHAQGYKGANVKVAVLDTGIHAAHPDLNVAGGASFVPSEPNATQDFQSHGTHVAGTIAALDNTIGVLGVAPSASLYAVKVLDRNGDGQYSWIISGIEWAVANNMDVINMSLGGPHSSTALKNAVDTANNRGVVVVAAAGNSGSTGSTSTVGYPAKYDSTIAVANVNSSNVRNSSSSAGPELDVSAPGTSILSTVPSSGYTCYTGTSMAAPHVAGAAALILSKNPNLSNSQVRQRLENTATPLGNSFYYGKGLINAEAASN

SEQ ID NO: 10 - protein, 275 aa, Artificial Sequence
  Mutationsvariante 8
AQTVPYGITQIKAPAVHAQGYKGANVKVAVLDTGIHAAHPDLNVAGGASFVPSEPNATQDFQSHGTHVAGTIAALDNTIGVLGVAPSASLYAVKVLDRNGDGQYSWIISGIEWAVANNMDVINMSLGGPDSSKALKNAVDTANNRGVVVVAAAGNSGSTGSTSTVGYPAKYDSTIAVANVNSSNVRNSSSSAGPELDVSAPGTSILSTVPSSGYTCYTGTSMAAPHVAGAAALILSKNPNLSNSQVRQRLENTATPLGNSFYYGKGLINAEAASN

SEQ ID NO: 11 - protein, 275 aa, Artificial Sequence
  Mutationsvariante 9
AQTVPYGITQIKAPAVHAQGYKGANVKVGVLDTGIHAAHPDLNVAGGASFVPSEPNATQDFQSHGTHVAGTIAALDNTIGVLGVAPSASLYAVKVLDRNGEGQYSWIISGIEWAVANNMDVINMSLGGPDKSTALKNAVDTANNRGVVVVAAAGNSGSTGSTSTVGYPAKYDSTIAVANVNSSNVRNSSSSAGPELDVSAPGTSILSTVPSSGYTCYTGTSMAAPHVAGAAALILSKNPNLSNSQVRQRLENTATPLGNSFYYGKGLINAEAASN

SEQ ID NO: 12 - protein, 275 aa, Artificial Sequence
  Mutationsvariante 10
AQTVPYGITQIKAPAVHAQGYKGANVKVAVLDTGIHAAHPDLNVAGGASFVPSEPNATQDFQSHGTHVAGTIAALDNTIGVLGVAPSASLYAVKVLDRNGDGQYSWIISGIEWAVANNMDVINMSLGGPDNSKALKNAVDTANLRGVVVVAAAGNSGSTGSTSTVGYPAKYDSTIAVANVNSSNVRNSSSSAGPELDVSAPGTSILSTVPSSGYTCYTGTSMASPHVAGAAALILSKNPNLSNSQVRQRLESTATPLGNSFYYGKGLINAEAASN

SEQ ID NO: 13 - protein, 275 aa, Artificial Sequence
  Mutationsvariante 11
AQTVPYGITQIKAPAVHAQGYKGANVKVAVLDTGIHAAHPDLNVAGGASFVPSEPNATQDFQSHGTHVAGTIAALDNTIGVLGVAPSASLYAVKVLDRNGDGQYSWIISGIEWAVANNMDVINMSLGGPNSSTALKNAVDTANKRGVVVVAAAGNSGSTGSTSTVGYPAKYDSTIAVANVNSSNVRNSSSSAGPELDVSAPGTSILSTVPSSGYTCYTGTSMATPHVAGAAALILSKNPNLSNSQVRQRLENTATPLGNSFYYGKGLINAEAASN

SEQ ID NO: 14 - protein, 275 aa, Artificial Sequence
  Mutationsvariante 12
AQTVPYGITQIKAPAVHAQGYKGANVKVAVLDTGIHAAHPDLNVAGGASFVPSEPNATQDFQSHGTHVAGTIAALDNTIGVLGVAPSASLYAVKVLDRNGEGQYSWIISGIEWAVANNMDVINMSLGGPDSSYALKNAVDTANARGVVVVAAAGNSGSTGSTSTVGYPAKYDSTIAVANVNSSNVRNSSSSAGPELDVSAPGTSILSTVPSSGYTCYTGTSMAAPHVAGAAALILSKNPNLSNSQVRQRLENTATPLGNSFYYGKGLINAEAASN

SEQ ID NO: 15 - protein, 275 aa, Artificial Sequence
  Mutationsvariante 13
AQTVPYGITQIKAPAVHAQGYKGANVKVGVLDTGIHAAHPDLNVAGGASFVPSEPNATQDFQSHGTHVAGTIAALDNTIGVLGVAPSASLYAVKVLDRNGEGQYSWIISGIEWAVANNMDVINMSLGGPSGSTALKNAVDTANNRGVVVVAAAGNSGSTGSTSTVGYPAKYDSTIAVANVNSSNVRNSSSSAGPELDVSAPGTSILSTVPSSGYTCYTGTSMATPHVAGAAALILSKNPNLSNSQVRQRLESTATPLGNSFYYGKGLINAEAASN

SEQ ID NO: 16 - protein, 275 aa, Artificial Sequence
  Mutationsvariante 14
AQTVPYGITQIKAPAVHAQGYKGANVKVAVLDTGIHAAHPDLNVAGGVSFVPSEPNATQDFQSHGTHVAGTIAALDNTIGVLGVAPSASLYAVKVLDRNGDGQYSWIISGIEWAVANNMDVINMSLGGPNSSRALKNAVDTANNRGVVVVAAAGNSGSTGSTSTVGYPAKYDSTIAVANVNSSNVRNSSSSAGPELDVSAPGTSILSTVPSSGYTCYTGTSMAAPHVAGAAALILSKNPNLSNSQVRQRLENTATPLGNSFYYGKGLINAEAASN

SEQ ID NO: 17 - protein, 275 aa, Artificial Sequence
  Mutationsvariante 15
AQTVPYGITQIKAPAVHAQGYKGANVKVAVLDTGIHAAHPDLNVAGGASFVPSEPNATQDFQSHGTHVAGTIAALDNTIGVLGVAPSASLYAVKVLDRNGDGQYSWIISGIEWAVANNMDVINMSLGGPNDSRALKNAVDTANNRGVVVVAAAGNSGSTGSTSTVGYPAKYDSTIAVANVNSSNVRNSSSSAGPELDVSAPGTSILSTVPSSGYTCYTGTSMAAPHVAGAAALILSKNPNLSNSQVRQRLENTATPLGNSFYYGKGLINAEAASN

SEQ ID NO: 18 - protein, 275 aa, Artificial Sequence
  Ausgangsmuitante 1
AQTVPYGITQIKAPAVHAQGYKGANVKVAVLDTGIHAAHPDLNVAGGASFVPSEPNATQDFQSHGTHVAGTIAALDNTIGVLGVAPSASLYAVKVLDRNGDGQYSWIISGIEWAVANNMDVINMSLGGPNGSTALKNAVDTANNRGVVVVAAAGNSGSTGSTSTVGYPAKYDSTIAVANVNSSNVRNSSSSAGPELDVSAPGTSILSTVPSSGYTCYTGTSMASPHVAGAAALILSKNPNLSNSQVRQRLENTATPLGNSFYYGKGLINAEAASN

SEQ ID NO: 19 - protein, 275 aa, Artificial Sequence
  Mutante 18
AQTVPYGITQIKAPAVHAQGYKGANVKVAVLDTGIHAAHPDLNVAGGASFVPSEPNATQDFQSHGTHVAGTIAALDNTIGVLGVAPSASLYAVKVLDRNGDGQYSWIISGIEWAVANNMDVINMSLGGPDGSTALKNAVDTANKRGVVVVAAAGNSGSTGSTSTVGYPAKYDSTIAVANVNSSNVRNSSSSAGPELDVSAPGTSILSTVPSSGYTSYTGTSMASPHVAGAAALILSKNPNLSNSQVRQRLETTATPLGNSFYYGKGLINAEAASN

SEQ ID NO: 20 - protein, 275 aa, Artificial Sequence
  Mutante 19
AQTVPYGITQIKAPAVHAQGYKGANVKVAVLDTGIHAAHPDLNVAGGASFVPSEPNATQDFQSHGTHVAGTIAALDNTIGVLGVAPSASLYAVKVLDRNGDGQYSWIISGIEWAVANNMDVINMSLGGPDGSTALKNAVDTANKRGVVVVAAAGNSGSTGSTSTVMYPAKYDSTIAVANVNSSNVRNSSSSAGPELDVSAPGTSILSTVPSSGYTSYTGTSMASPHVAGAAALILSKNPNLSNSQVRQRLETTATPLGNSFYYGKGLINAEAASN

SEQ ID NO: 21 - protein, 275 aa, Artificial Sequence
  Mutante 20
AQTVPYGITQIKAPAVHAQGYKGANVKVAVLDTGIHAAHPDLNVAGGASFVPSEPNATQDFQSHGTHVAGTIAALDNTIGVLGVAPSASLYAVKVLDRNGDGQYSWIISGIEWAVANNMDVINMSLGGPDGSTALKNAVDTANKRGVVVVAAAGNSGSTGSTSTVQYPAKYDSTIAVANVNSSNVRNSSSSAGPELDVSAPGTSILSTVPSSGYTSYTGTSMASPHVAGAAALILSKNPNLSNSQVRQRLETTATPLGNSFYYGKGLINAEAASN

SEQ ID NO: 22 - protein, 275 aa, Artificial Sequence
  Mutante 21
AQTVPYGITQIKAPAVHAQGYKGANVKVAVLDTGIHAAHPDLNVAGGASFVPSEPNATQDFQSHGTHVAGTIAALDNTIGVLGVAPSASLYAVKVLDRNGDGQYSWIISGIEWAVANNMDVINMSLGGPDGSTALKNAVDTANKRGVVVVAAAGNSGSTGSTSTVAYPAKYDSTIAVANVNSSNVRNSSSSAGPELDVSAPGTSILSTVPSSGYTSYTGTSMASPHVAGAAALILSKNPNLSNSQVRQRLETTATPLGNSFYYGKGLINAEAASN

SEQ ID NO: 23 - protein, 275 aa, Artificial Sequence
  Mutante 22
AQTVPYGITQIKAPAVHAQGYKGANVKVAVLDTGIHAAHPDLNVAGGASFVPSEPNATQDFQSHGTHVAGTIAALDNTIGVLGVAPSASLYAVKVLDRNGDGQYSWIISGIEWAVANNMDVINMSLGGPDGSTALKNAVDTANKRGVVVVAAAGNSGSTGSTSTVGYPAKYDSTIAVANVNSSNVRNSSSSAGPELDVSAPGTSILSTVPSSGYTSMTGTSMASPHVAGAAALILSKNPNLSNSQVRQRLETTATPLGNSFYYGKGLINAEAASN

SEQ ID NO: 24 - protein, 275 aa, Artificial Sequence
  Mutante 23
AQTVPYGITQIKAPAVHAQGYKGANVKVAVLDTGIHAAHPDLNVAGGASFVPSEPNATQDFQSHGTHVAGTIAALDNTIGVLGVAPSASLYAVKVLDRNGDGQYSWIISGIEWAVANNMDVINMSLGGPDGSTALKNAVDTANKRGVVVVAAAGNGGSTGSTSTVGYPAKYDSTIAVANVNSSNVRNSSSSAGPELDVSAPGTSILSTVPSSGYTSYTGTSMASPHVAGAAALILSKNPNLSNSQVRQRLETTATPLGNSFYYGKGLINAEAASN